European Patent Application EP 4 686 478 A1, published February 4, 2026. Title: QBP1 FOR USE IN THE TREATMENT AND/OR PREVENTION OF TYPE 2 DIABETES. Applicant: Consejo Superior de Investigaciones Cientificas (CSIC). Application EP. The sequence listing filed with the application follows.

SEQUENCE LISTING (5 sequences)

SEQ ID NO: 1 - protein, 8 aa, synthetic construct
WKWWPGIF

SEQ ID NO: 2 - protein, 11 aa, synthetic construct
SNWKWWPGIFD

SEQ ID NO: 3 - protein, 16 aa, synthetic construct
RQIKIWFQNRRMKWKK

SEQ ID NO: 4 - protein, 11 aa, synthetic construct
YGRKKRRQRRR

SEQ ID NO: 5 - protein, 26 aa, synthetic construct
RQIKIWFQNRRMKWKKGGWKWWPGIF